European Patent Application EP 4 275 702 A2, published November 15, 2023. Title: CD70 COMBINATION THERAPY. Applicant: argenx BVBA. Application EP 23177089.2, filed January 16, 2019. The sequence listing filed with the application follows.

SEQUENCE LISTING (136 sequences)

SEQ ID NO: 1 - protein, 5 aa, synthetic construct
  REGION 1..5: note = Synthetic peptide
VYYMN

SEQ ID NO: 2 - protein, 17 aa, synthetic construct
  REGION 1..17: note = Synthetic peptide
DINNEGGTTYYADSVKG

SEQ ID NO: 3 - protein, 13 aa, synthetic construct
  REGION 1..13: note = Synthetic peptide
DAGYSNHVPIFDS

SEQ ID NO: 4 - protein, 122 aa, synthetic construct
  REGION 1..122: note = Synthetic peptide
EVQLVESGGGLVQPGGSLRLSCAASGFTFSVYYMNWVRQAPGKGLEWVSDINNEGGTTYYADSVKGRFTISRDNSKNSLYLQMNSLRAEDTAVYYCARDAGYSNHVPIFDSWGQGTLVTVSS

SEQ ID NO: 5 - protein, 14 aa, synthetic construct
  REGION 1..14: note = Synthetic peptide
GLKSGSVTSDNFPT

SEQ ID NO: 6 - protein, 7 aa, synthetic construct
  REGION 1..7: note = Synthetic peptide
NTNTRHS

SEQ ID NO: 7 - protein, 10 aa, synthetic construct
  REGION 1..10: note = Synthetic peptide
ALFISNPSVE

SEQ ID NO: 8 - protein, 111 aa, synthetic construct
  REGION 1..111: note = Synthetic peptide
QAVVTQEPSLTVSPGGTVTLTCGLKSGSVTSDNFPTWYQQTPGQAPRLLIYNTNTRHSGVPDRFSGSILGNKAALTITGAQADDEAEYFCALFISNPSVEFGGGTQLTVLG

SEQ ID NO: 9 - protein, 123 aa, synthetic construct
  REGION 1..123: note = Synthetic peptide
EVQLVESGGGLVQPGGSLRLSCAASGFTFSSYAMSWVRQAPGKGPEWVSHINSGGGNTKYADSVKGRFTISRDNAKNTLYLQMNTLKPEDTAVYYCAKDVSGGYYGTYALDAWGQGTQVVVSS

SEQ ID NO: 10 - protein, 106 aa, synthetic construct
  REGION 1..106: note = Synthetic peptide
SYELTQSPSVSVALKQTAKITCGGDNIGSKSAQWYQQKPGQAPVLVIYADSRRPSGIPERFSGSNSGNTATLTISGAQAEDEADYYCQVWDSSAAVFGGGTHLTVL

SEQ ID NO: 11 - protein, 121 aa, synthetic construct
  REGION 1..121: note = Synthetic peptide
EVQVQESGGGLVQPGGSLRLSCAASGFTFSSYAMSWVRQAPGKGLEWVSDINSGGGSTVYTDSVKGRFTISRDNAKNTLYLQMNSLKPDDTAVYYCATGGSYYSYRLFDYWGQGTQVTVSS

SEQ ID NO: 12 - protein, 114 aa, synthetic construct
  REGION 1..114: note = Synthetic peptide
DIQMTQSPSSVIVSAGEKVTINCKSSQSVLDSSNQKNYLAWYQQRLGQSPRLLIYWASTRESGVPDRFSGSGSTTDFTLTISSFQPEDAAVYYCQQGYSVPVTFGQGTKVELKR

SEQ ID NO: 13 - protein, 124 aa, synthetic construct
  REGION 1..124: note = Synthetic peptide
QVQLVESGGGLVQPGGSLRLSCAASGFTFSNYWMYWVRQAPGKGLEWVSTINTNGAITLYADNVKDRFTVSRDNAKNTLYLQMNSLKSEDTAVYYCAKVKLSGYPHPYYAMDYWGKGTLVTVSS

SEQ ID NO: 14 - protein, 115 aa, synthetic construct
  REGION 1..115: note = Synthetic peptide
NFMLTQPPSLSGSLGQSARLTCTLGSGNSIGAHTISWYQQKAGSPPRYLLNYYSDSSNHQASGVPSRFSGSKDDSTNAGLLLISGLQPEDEADYYCAAGDGSGTVFGGGTKLTVL

SEQ ID NO: 15 - protein, 122 aa, synthetic construct
  REGION 1..122: note = Synthetic peptide
QVQLVESGPGLVKPSQTLSLTCTVSGGSITTSDDAWSWIRQPAGKGLEWMGVIAYDGSTRYSPSLQSRTSISRDTSKNQFSLQLSSVTPEDTAVYYCARTKGVGGTWALDAWGQGTLVTVSS

SEQ ID NO: 16 - protein, 114 aa, synthetic construct
  REGION 1..114: note = Synthetic peptide
EIVLTQSPSSVTASVGEKVTINCKSSQSVLSSSNQKNYLSWYQQRLGQSPRLLITWASTRESGVPDRFSGSGSTTDFTLTISSFQPEDAAVYYCQQGYGAPLTFGQGTKVELKR

SEQ ID NO: 17 - protein, 122 aa, synthetic construct
  REGION 1..122: note = Synthetic peptide
QVQLVESGGGLVQPGGSLRLSCAASGFAFSSYDMSWVRQAPGKGLEWVSTINSGGGSTNYADSMKGRFTISRDNAKNTVYLQMNSLKPEDTAVYYCAARSPYYTRVPLYDYWGQGTQVTVSS

SEQ ID NO: 18 - protein, 110 aa, synthetic construct
  REGION 1..110: note = Synthetic peptide
QAVVTQEPSLSVSLGGTVTLTCGLRSGSVTTSNYPGWFKQTPGQAPRTLIFGASSRHSGVPSRYSGSISGNKAALTITGAEPEDEADYYCALNKGTYTDVFGGGTKLTVL

SEQ ID NO: 19 - protein, 125 aa, synthetic construct
  REGION 1..125: note = Synthetic peptide
EVQLQESGPGLVKPSQTLSLTCTVSGASVTTRYNYWSWIRQPPGKGLEWMGAITYSGSTYYSPSLKSRTSISRDTSKNQFTLQLSSVTPEDTAVYYCATEGSSSTGVSRYSFGSWGQGTQVTVSS

SEQ ID NO: 20 - protein, 111 aa, synthetic construct
  REGION 1..111: note = Synthetic peptide
ATMLTQSPGSLSVVPGESASISCKASQSLTHTDGTTALYWLQQKPGQRPQLLIYEVSVRASGVPDRFTGSGSGSDFTLKINGVKAEDAGVYYCAQVAYYPTFGQGTKVELK

SEQ ID NO: 21 - protein, 118 aa, synthetic construct
  REGION 1..118: note = Synthetic peptide
QVQLQESGPGLVKPSQTLSLTCTVSGGSITTNRYLWTWIRQTPGKGLEWVGAIAYSGRTYYSPSLKSRTSISRDTSKNQFTLQLSSVTPEDTGVYYCAHFTGWGGYYWGQGTQVTVSS

SEQ ID NO: 22 - protein, 110 aa, synthetic construct
  REGION 1..110: note = Synthetic peptide
QSALTQPPSVSGTLGKTVTISCAGTSSDIGGYNSVSWYQQLPGTAPKLLIYEVNKRASGIPDRFSGSKSGNTASLSISGLQSEDEADYYCASYRSANNVVFGGGTKLTVL

SEQ ID NO: 23 - protein, 122 aa, synthetic construct
  REGION 1..122: note = Synthetic peptide
QVQLVESGGGLVQPGGSLRLSCAASGFAFSSYDMSWVRQAPGKGPEWVSTINSGGGSTSYADSVKGRFTISRDNAKNTVYLQMNSLKPEDTAVYYCAARSLYYTRVPMYDYWGQGTQVTVSK

SEQ ID NO: 24 - protein, 110 aa, synthetic construct
  REGION 1..110: note = Synthetic peptide
QAVVTQEPSLSVSPGGTVTLTCGLSSGSVTTNNYPGWFQQTPGQAPRTLIYSTSSRHSGVPSRFSGSISGNKAALTITGAQPEDEADYYCALDIGSYTAVFGGGTHLTVL

SEQ ID NO: 25 - protein, 125 aa, synthetic construct
  REGION 1..125: note = Synthetic peptide
EVQLVQPGAELRNPGASVKVSCKASGYTFTMYYIDWVRQAPGQGLEWMGRIDPEDGGTKYAQKFQGRVTFTADTSTSTAYVELSSLRSEDTAVYYCARIPNGGSYYYTPYDYDYWGQGTQVTVSS

SEQ ID NO: 26 - protein, 110 aa, synthetic construct
  REGION 1..110: note = Synthetic peptide
QAVVTQEPSLSVSPGGTVTLTCGLTSGSVTSSNYPGWYRQTPGQAPRPLIYNTNSRHPGVPSRYSGSISENKATLTITGAEPEDEADYYCALHKGSYTAVFGGGTHLTVL

SEQ ID NO: 27 - protein, 121 aa, synthetic construct
  REGION 1..121: note = Synthetic peptide
QVQLQESGGGLVQPGGSLTLSCAASGFFFSSYAMSWVRQAPGKGLEWVSSISAGGGTSYYADSVKGRFTISRDSAKNTLVLQMNSLKPEDTAVYYCAKKRQNFWSEGYDSWGQGTQVTVSS

SEQ ID NO: 28 - protein, 110 aa, synthetic construct
  REGION 1..110: note = Synthetic peptide
HSAVTQPPSVSGSPGKAVTISCVGSSSDVGYGDYVSWYQQLPGMAPKLLIYDVEKRASGIPDRFSGSKSGNTASLTISGLQSEDEADYYCASYRSDSNFVFGGGTHLAVL

SEQ ID NO: 29 - protein, 120 aa, synthetic construct
  REGION 1..120: note = Synthetic peptide
QLQLVESGGGLVQPGGSLRLSCAASGFTFGSYDMSWVRQAPGKGPEWVSRITSGGGSTYADSVKGRFTISRDNAKNTLSLQMNSLKSEDTAVYYCAAGQYSDGYYPYDYWGQGTQVTVSS

SEQ ID NO: 30 - protein, 107 aa, synthetic construct
  REGION 1..107: note = Synthetic peptide
DIVMTQSPSSLSASLGDRVTITCQASQSISSYLAWYQQKPGQGPKLLIYGASRLEPGVPSRFSGSGSGTSFTLTISGVEAEDLATYYCLQDYSWPYSFGSGTRLEIK

SEQ ID NO: 31 - protein, 114 aa, synthetic construct
  REGION 1..114: note = Synthetic peptide
ELQVVESGGGLVQPGGSLRLSCAASGFTFGSYDMSWHRQAPRKGPEWVSTISAGGGRTYYADSVKGRFTISRDNAKNTLYLQMNSLKPEDTAVYFCTKIVLDSWGQGTQVTVSS

SEQ ID NO: 32 - protein, 111 aa, synthetic construct
  REGION 1..111: note = Synthetic peptide
DVVLTQTPGSLSVVPGESASISCKASQSLIHIDGKTYLYWLLQKPGRRPELLIYQVSNHESGVPDRFTGSGSGTDFTLKISGVKAEDAGVYYCAQATYYPSFGSGTRLEIK

SEQ ID NO: 33 - protein, 117 aa, synthetic construct
  REGION 1..117: note = Synthetic peptide
EVQLVESGGGLVQPGGSLRLSCAASGFTFDDYTMSWVRQVPGKGLEWISGISGNGGRTDYVEPIEGRFTISRDNAKNTLYLQMNSLKSEDTAVYYCAKTSPQSLDYWGQGTQVTVSS

SEQ ID NO: 34 - protein, 113 aa, synthetic construct
  REGION 1..113: note = Synthetic peptide
DIVMTQSPSSVTASVGEKVTINCKSSQSVVSGSNQKSYLNWYQQRPGQPPRLLIYYASTQESGIPDRFSGSGSTTDFTLTISSVQPEDAAVYYCQQAYSAPYNFGSGTRLEIK

SEQ ID NO: 35 - protein, 114 aa, synthetic construct
  REGION 1..114: note = Synthetic peptide
EVQLVESGGGLVQPGGSLRLSCAASGFTFGSYDMSWVRQAPGKGPEWVSTISAGGGRTYYADSVKDRFTISRDNAKNTLYLQMNSLKPEDTAVYYCAKVVIDYWGQGTQVTVSS

SEQ ID NO: 36 - protein, 111 aa, synthetic construct
  REGION 1..111: note = Synthetic peptide
DVVLTQTPGSLSVVPGESASISCKASQSLVHTDGKTYVYWLLQKPGQRPHLLIYQVSNHESGVPDRFTGSGSGTDFTLKISGVKAEDAGVYYCAQATYYPSFGSGTRLEIK

SEQ ID NO: 37 - protein, 125 aa, synthetic construct
  REGION 1..125: note = Synthetic peptide
EVQLVESGGGLVQPGGSLRLSCAASGFTFSSYSMSWVRQAPGKGPEWVSGINTSGGTTSYAASVKGRFTVSRDNAKNTLSLQMNSLEPEDTAVYYCVKHIRWSGSNYYYYGMDYWGKGTLVTVSS

SEQ ID NO: 38 - protein, 110 aa, synthetic construct
  REGION 1..110: note = Synthetic peptide
QAVLTQPPSVSGSPGQRFTISCTGSNRNIGNNYVNWYQQLPGTAPKLLIYSDNLRTSGVPARFSASKSGTTSSLTISGLQAEDEAVYYCSSWDDSLSGAVFGGGTHLTVL

SEQ ID NO: 39 - protein, 5 aa, synthetic construct
  REGION 1..5: note = Synthetic peptide
SYAMS

SEQ ID NO: 40 - protein, 17 aa, synthetic construct
  REGION 1..17: note = Synthetic peptide
HINSGGGNTKYADSVKG

SEQ ID NO: 41 - protein, 14 aa, synthetic construct
  REGION 1..14: note = Synthetic peptide
DVSGGYYGTYALDA

SEQ ID NO: 42 - protein, 17 aa, synthetic construct
  REGION 1..17: note = Synthetic peptide
DINSGGGSTVYTDSVKG

SEQ ID NO: 43 - protein, 12 aa, synthetic construct
  REGION 1..12: note = Synthetic peptide
GGSYYSYRLFDY

SEQ ID NO: 44 - protein, 5 aa, synthetic construct
  REGION 1..5: note = Synthetic peptide
NYWMY

SEQ ID NO: 45 - protein, 17 aa, synthetic construct
  REGION 1..17: note = Synthetic peptide
TINTNGAITLYADNVKD

SEQ ID NO: 46 - protein, 15 aa, synthetic construct
  REGION 1..15: note = Synthetic peptide
VKLSGYPHPYYAMDY

SEQ ID NO: 47 - protein, 7 aa, synthetic construct
  REGION 1..7: note = Synthetic peptide
TSDDAWS

SEQ ID NO: 48 - protein, 16 aa, synthetic construct
  REGION 1..16: note = Synthetic peptide
VIAYDGSTRYSPSLQS

SEQ ID NO: 49 - protein, 12 aa, synthetic construct
  REGION 1..12: note = Synthetic peptide
TKGVGGTWALDA

SEQ ID NO: 50 - protein, 5 aa, synthetic construct
  REGION 1..5: note = Synthetic peptide
SYDMS

SEQ ID NO: 51 - protein, 17 aa, synthetic construct
  REGION 1..17: note = Synthetic peptide
TINSGGGSTNYADSMKG

SEQ ID NO: 52 - protein, 13 aa, synthetic construct
  REGION 1..13: note = Synthetic peptide
RSPYYTRVPLYDY

SEQ ID NO: 53 - protein, 7 aa, synthetic construct
  REGION 1..7: note = Synthetic peptide
TRYNYWS

SEQ ID NO: 54 - protein, 16 aa, synthetic construct
  REGION 1..16: note = Synthetic peptide
AITYSGSTYYSPSLKS

SEQ ID NO: 55 - protein, 15 aa, synthetic construct
  REGION 1..15: note = Synthetic peptide
EGSSSTGVSRYSFGS

SEQ ID NO: 56 - protein, 7 aa, synthetic construct
  REGION 1..7: note = Synthetic peptide
TNRYLWT

SEQ ID NO: 57 - protein, 16 aa, synthetic construct
  REGION 1..16: note = Synthetic peptide
AIAYSGRTYYSPSLKS

SEQ ID NO: 58 - protein, 8 aa, synthetic construct
  REGION 1..8: note = Synthetic peptide
FTGWGGYY

SEQ ID NO: 59 - protein, 17 aa, synthetic construct
  REGION 1..17: note = Synthetic peptide
TINSGGGSTSYADSVKG

SEQ ID NO: 60 - protein, 13 aa, synthetic construct
  REGION 1..13: note = Synthetic peptide
RSLYYTRVPMYDY

SEQ ID NO: 61 - protein, 5 aa, synthetic construct
  REGION 1..5: note = Synthetic peptide
MYYID

SEQ ID NO: 62 - protein, 17 aa, synthetic construct
  REGION 1..17: note = Synthetic peptide
RIDPEDGGTKYAQKFQG

SEQ ID NO: 63 - protein, 16 aa, synthetic construct
  REGION 1..16: note = Synthetic peptide
IPNGGSYYYTPYDYDY

SEQ ID NO: 64 - protein, 17 aa, synthetic construct
  REGION 1..17: note = Synthetic peptide
SISAGGGTSYYADSVKG

SEQ ID NO: 65 - protein, 12 aa, synthetic construct
  REGION 1..12: note = Synthetic peptide
KRQNFWSEGYDS

SEQ ID NO: 66 - protein, 16 aa, synthetic construct
  REGION 1..16: note = Synthetic peptide
RITSGGGSTYADSVKG

SEQ ID NO: 67 - protein, 12 aa, synthetic construct
  REGION 1..12: note = Synthetic peptide
GQYSDGYYPYDY

SEQ ID NO: 68 - protein, 17 aa, synthetic construct
  REGION 1..17: note = Synthetic peptide
TISAGGGRTYYADSVKG

SEQ ID NO: 69 - protein, 5 aa, synthetic construct
  REGION 1..5: note = Synthetic peptide
IVLDS

SEQ ID NO: 70 - protein, 5 aa, synthetic construct
  REGION 1..5: note = Synthetic peptide
DYTMS

SEQ ID NO: 71 - protein, 5 aa, synthetic construct
  REGION 1..5: note = Synthetic peptide
DYTMS

SEQ ID NO: 72 - protein, 17 aa, synthetic construct
  REGION 1..17: note = Synthetic peptide
GISGNGGRTDYVEPIEG

SEQ ID NO: 73 - protein, 8 aa, synthetic construct
  REGION 1..8: note = Synthetic peptide
TSPQSLDY

SEQ ID NO: 74 - protein, 5 aa, synthetic construct
  REGION 1..5: note = Synthetic peptide
VVIDY

SEQ ID NO: 75 - protein, 5 aa, synthetic construct
  REGION 1..5: note = Synthetic peptide
SYSMS

SEQ ID NO: 76 - protein, 17 aa, synthetic construct
  REGION 1..17: note = Synthetic peptide
GINTSGGTTSYAASVKG

SEQ ID NO: 77 - protein, 16 aa, synthetic construct
  REGION 1..16: note = Synthetic peptide
HIRWSGSNYYYYGMDY

SEQ ID NO: 78 - protein, 11 aa, synthetic construct
  REGION 1..11: note = Synthetic peptide
GGDNIGSKSAQ

SEQ ID NO: 79 - protein, 7 aa, synthetic construct
  REGION 1..7: note = Synthetic peptide
ADSRRPS

SEQ ID NO: 80 - protein, 9 aa, synthetic construct
  REGION 1..9: note = Synthetic peptide
QVWDSSAAV

SEQ ID NO: 81 - protein, 17 aa, synthetic construct
  REGION 1..17: note = Synthetic peptide
KSSQSVLDSSNQKNYLA

SEQ ID NO: 82 - protein, 7 aa, synthetic construct
  REGION 1..7: note = Synthetic peptide
WASTRES

SEQ ID NO: 83 - protein, 9 aa, synthetic construct
  REGION 1..9: note = Synthetic peptide
QQGYSVPVT

SEQ ID NO: 84 - protein, 14 aa, synthetic construct
  REGION 1..14: note = Synthetic peptide
TLGSGNSIGAHTIS

SEQ ID NO: 85 - protein, 13 aa, synthetic construct
  REGION 1..13: note = Synthetic peptide
YYSDSSNHQASGV

SEQ ID NO: 86 - protein, 9 aa, synthetic construct
  REGION 1..9: note = Synthetic peptide
AAGDGSGTV

SEQ ID NO: 87 - protein, 17 aa, synthetic construct
  REGION 1..17: note = Synthetic peptide
KSSQSVLSSSNQKNYLS

SEQ ID NO: 88 - protein, 9 aa, synthetic construct
  REGION 1..9: note = Synthetic peptide
QQGYGAPLT

SEQ ID NO: 89 - protein, 14 aa, synthetic construct
  REGION 1..14: note = Synthetic peptide
GLRSGSVTTSNYPG

SEQ ID NO: 90 - protein, 7 aa, synthetic construct
  REGION 1..7: note = Synthetic peptide
GASSRHS

SEQ ID NO: 91 - protein, 10 aa, synthetic construct
  REGION 1..10: note = Synthetic peptide
ALNKGTYTDV

SEQ ID NO: 92 - protein, 16 aa, synthetic construct
  REGION 1..16: note = Synthetic peptide
KASQSLTHTDGTTALY

SEQ ID NO: 93 - protein, 7 aa, synthetic construct
  REGION 1..7: note = Synthetic peptide
EVSVRAS

SEQ ID NO: 94 - protein, 8 aa, synthetic construct
  REGION 1..8: note = Synthetic peptide
AQVAYYPT

SEQ ID NO: 95 - protein, 14 aa, synthetic construct
  REGION 1..14: note = Synthetic peptide
AGTSSDIGGYNSVS

SEQ ID NO: 96 - protein, 7 aa, synthetic construct
  REGION 1..7: note = Synthetic peptide
EVNKRAS

SEQ ID NO: 97 - protein, 10 aa, synthetic construct
  REGION 1..10: note = Synthetic peptide
ASYRSANNVV

SEQ ID NO: 98 - protein, 14 aa, synthetic construct
  REGION 1..14: note = Synthetic peptide
GLSSGSVTTNNYPG

SEQ ID NO: 99 - protein, 7 aa, synthetic construct
  REGION 1..7: note = Synthetic peptide
STSSRHS

SEQ ID NO: 100 - protein, 10 aa, synthetic construct
  REGION 1..10: note = Synthetic peptide
ALDIGSYTAV

SEQ ID NO: 101 - protein, 14 aa, synthetic construct
  REGION 1..14: note = Synthetic peptide
GLTSGSVTSSNYPG

SEQ ID NO: 102 - protein, 7 aa, synthetic construct
  REGION 1..7: note = Synthetic peptide
NTNSRHP

SEQ ID NO: 103 - protein, 10 aa, synthetic construct
  REGION 1..10: note = Synthetic peptide
ALHKGSYTAV

SEQ ID NO: 104 - protein, 14 aa, synthetic construct
  REGION 1..14: note = Synthetic peptide
VGSSSDVGYGDYVS

SEQ ID NO: 105 - protein, 7 aa, synthetic construct
  REGION 1..7: note = Synthetic peptide
DVEKRAS

SEQ ID NO: 106 - protein, 10 aa, synthetic construct
  REGION 1..10: note = Synthetic peptide
ASYRSDSNFV

SEQ ID NO: 107 - protein, 11 aa, synthetic construct
  REGION 1..11: note = Synthetic peptide
QASQSISSYLA

SEQ ID NO: 108 - protein, 7 aa, synthetic construct
  REGION 1..7: note = Synthetic peptide
GASRLEP

SEQ ID NO: 109 - protein, 9 aa, synthetic construct
  REGION 1..9: note = Synthetic peptide
LQDYSWPYS

SEQ ID NO: 110 - protein, 16 aa, synthetic construct
  REGION 1..16: note = Synthetic peptide
KASQSLIHIDGKTYLY

SEQ ID NO: 111 - protein, 7 aa, synthetic construct
  REGION 1..7: note = Synthetic peptide
QVSNHES

SEQ ID NO: 112 - protein, 8 aa, synthetic construct
  REGION 1..8: note = Synthetic peptide
AQATYYPS

SEQ ID NO: 113 - protein, 17 aa, synthetic construct
  REGION 1..17: note = Synthetic peptide
KSSQSVVSGSNQKSYLN

SEQ ID NO: 114 - protein, 7 aa, synthetic construct
  REGION 1..7: note = Synthetic peptide
YASTQES

SEQ ID NO: 115 - protein, 9 aa, synthetic construct
  REGION 1..9: note = Synthetic peptide
QQAYSAPYN

SEQ ID NO: 116 - protein, 16 aa, synthetic construct
  REGION 1..16: note = Synthetic peptide
KASQSLVHTDGKTYVY

SEQ ID NO: 117 - protein, 8 aa, synthetic construct
  REGION 1..8: note = Synthetic peptide
AQATYYPS

SEQ ID NO: 118 - protein, 13 aa, synthetic construct
  REGION 1..13: note = Synthetic peptide
TGSNRNIGNNYVN

SEQ ID NO: 119 - protein, 7 aa, synthetic construct
  REGION 1..7: note = Synthetic peptide
SDNLRTS

SEQ ID NO: 120 - protein, 11 aa, synthetic construct
  REGION 1..11: note = Synthetic peptide
SSWDDSLSGAV

SEQ ID NO: 121 - protein, 117 aa, synthetic construct
  REGION 1..117: note = Synthetic peptide
QVQLVESGGGLVQPGGSLRLSCAASGFIFINYGMHWVRQAPGKGLEWVSAVNSGGASTDYADSVKGRFTISRDDAKNTLYLQMNSLKSEDTAVYYCVKGWFYGIHYWGKGTLVTVSS

SEQ ID NO: 122 - protein, 111 aa, synthetic construct
  REGION 1..111: note = Synthetic peptide
QAVLTQLPSVSGSPGQKITISCTGSSSNIGGGYSVQWFQHLPGTPPKLLIYGNSNRASGVPDRFSGSKSGSSASLTITGLQAEDEADYYCESYDDWLKGRGFGGGSKLTVL

SEQ ID NO: 123 - protein, 124 aa, synthetic construct
  REGION 1..124: note = Synthetic peptide
QVQLVESGPGLVKPSQTLSLTCTVSGGSITTNYYSWIWIRQPPGKGLEWMGASVYSGSTFYSPSLKNTSISKDTAQNQFTLQLRSVTPEDTAVYYCARASSAHWGSSFISIDYWGQGTQVTVSS

SEQ ID NO: 124 - protein, 110 aa, synthetic construct
  REGION 1..110: note = Synthetic peptide
QSVLTQPPSVSGSPGKTVTISCAGTSSDVGYGNYVSWYQQLPGMAPKLLIYDVDIRASGIADRFSGSKSGNTASLTISGLQSEDEADYYCASYRTNNNAVFGGGTHLTVL

SEQ ID NO: 125 - protein, 5 aa, synthetic construct
  REGION 1..5: note = Synthetic peptide
NYGMH

SEQ ID NO: 126 - protein, 17 aa, synthetic construct
  REGION 1..17: note = Synthetic peptide
AVNSGGASTDYADSVKG

SEQ ID NO: 127 - protein, 8 aa, synthetic construct
  REGION 1..8: note = Synthetic peptide
GWFYGIHY

SEQ ID NO: 128 - protein, 7 aa, synthetic construct
  REGION 1..7: note = Synthetic peptide
TNYYSWI

SEQ ID NO: 129 - protein, 16 aa, synthetic construct
  REGION 1..16: note = Synthetic peptide
ASVYSGSTFYSPSLKN

SEQ ID NO: 130 - protein, 15 aa, synthetic construct
  REGION 1..15: note = Synthetic peptide
ASSAHWGSSFISIDY

SEQ ID NO: 131 - protein, 14 aa, synthetic construct
  REGION 1..14: note = Synthetic peptide
TGSSSNIGGGYSVQ

SEQ ID NO: 132 - protein, 7 aa, synthetic construct
  REGION 1..7: note = Synthetic peptide
GNSNRAS

SEQ ID NO: 133 - protein, 11 aa, synthetic construct
  REGION 1..11: note = Synthetic peptide
ESYDDWLKGRG

SEQ ID NO: 134 - protein, 14 aa, synthetic construct
  REGION 1..14: note = Synthetic peptide
AGTSSDVGYGNYVS

SEQ ID NO: 135 - protein, 7 aa, synthetic construct
  REGION 1..7: note = Synthetic peptide
DVDIRAS

SEQ ID NO: 136 - protein, 10 aa, synthetic construct
  REGION 1..10: note = Synthetic peptide
ASYRTNNNAV